European Patent Application EP 4 484 444 A1, published January 1, 2025. Title: Protein and frangement thereof, and their use. Applicant: Centre National de la Recherche Scientifique. Application EP. The sequence listing filed with the application follows.

SEQUENCE LISTING (64 sequences)

SEQ ID NO: 1 - protein, 112 aa, Unidentified
CGGILTGESGFIGSEGFPGVYPPNSKCTWKITVPEGKVVVLNFRFIDLESDNLCRYDFVDVYNGHANGQRIGRFCGTFRPGALVSSGNKMMVQMISDANTAGNGFMAMFSAA

SEQ ID NO: 2 - protein, 392 aa, Homo sapiens
QSPERPVFTCGGILTGESGFIGSEGFPGVYPPNSKCTWKITVPEGKVVVLNFRFIDLESDNLCRYDFVDVYNGHANGQRIGRFCGTFRPGALVSSGNKMMVQMISDANTAGNGFMAMFSAAEPNERGDQYCGGLLDRPSGSFKTPNWPDRDYPAGVTCVWHIVAPKNQLIELKFEKFDVERDNYCRYDYVAVFNGGEVNDARRIGKYCGDSPPAPIVSERNELLIQFLSDLSLTADGFIGHYIFRPKKLPTTTEQPVTTTFPVTTGLKPTVALCQQKCRRTGTLEGNYCSSDFVLAGTVITTITRDGSLHATVSIINIYKEGNLAIQQAGKNMSARLTVVCKQCPLLRRGLNYIIMGQVGEDGRGKIMPNSFIMMFKTKNQKLLDALKNKQC

SEQ ID NO: 3 - protein, 415 aa, Homo sapiens
MRGANAWAPLCLLLAAATQLSRQQSPERPVFTCGGILTGESGFIGSEGFPGVYPPNSKCTWKITVPEGKVVVLNFRFIDLESDNLCRYDFVDVYNGHANGQRIGRFCGTFRPGALVSSGNKMMVQMISDANTAGNGFMAMFSAAEPNERGDQYCGGLLDRPSGSFKTPNWPDRDYPAGVTCVWHIVAPKNQLIELKFEKFDVERDNYCRYDYVAVFNGGEVNDARRIGKYCGDSPPAPIVSERNELLIQFLSDLSLTADGFIGHYIFRPKKLPTTTEQPVTTTFPVTTGLKPTVALCQQKCRRTGTLEGNYCSSDFVLAGTVITTITRDGSLHATVSIINIYKEGNLAIQQAGKNMSARLTVVCKQCPLLRRGLNYIIMGQVGEDGRGKIMPNSFIMMFKTKNQKLLDALKNKQC

SEQ ID NO: 4 - protein, 115 aa, Unidentified
CGGLLDRPSGSFKTPNWPDRDYPAGVTCVWHIVAPKNQLIELKFEKFDVERDNYCRYDYVAVFNGGEVNDARRIGKYCGDSPPAPIVSERNELLIQFLSDLSLTADGFIGHYIFR

SEQ ID NO: 5 - protein, 9 aa, Unidentified
EPNERGDQY

SEQ ID NO: 6 - protein, 9 aa, Unidentified
ATSGTEHQF

SEQ ID NO: 7 - protein, 419 aa, Unidentified
ETGHHHHHHLEVLFQGPASQSPERPVFTCGGILTGESGFIGSEGFPGVYPPNSKCTWKITVPEGKVVVLNFRFIDLESDNLCRYDFVDVYNGHANGQRIGRFCGTFRPGALVSSGNKMMVQMISDANTAGNGFMAMFSAAEPNERGDQYCGGLLDRPSGSFKTPNWPDRDYPAGVTCVWHIVAPKNQLIELKFEKFDVERDNYCRYDYVAVFNGGEVNDARRIGKYCGDSPPAPIVSERNELLIQFLSDLSLTADGFIGHYIFRPKLEVLFQGPKLPTTTEQPVTTTFPVTTGLKPTVALCQQKCRRTGTLEGNYCSSDFVLAGTVITTITRDGSLHATVSIINIYKEGNLAIQQAGKNMSARLTVVCKQCPLLRRGLNYIIMGQVGEDGRGKIMPNSFIMMFKTKNQKLLDALKNKQC

SEQ ID NO: 8 - protein, 257 aa, Unidentified
GPASQSPERPVFTCGGILTGESGFIGSEGFPGVYPPNSKCTWKITVPEGKVVVLNFRFIDLESDNLCRYDFVDVYNGHANGQRIGRFCGTFRPGALVSSGNKMMVQMISDANTAGNGFMAMFSAAEPNERGDQYCGGLLDRPSGSFKTPNWPDRDYPAGVTCVWHIVAPKNQLIELKFEKFDVERDNYCRYDYVAVFNGGEVNDARRIGKYCGDSPPAPIVSERNELLIQFLSDLSLTADGFIGHYIFRPKLEVLFQ

SEQ ID NO: 9 - protein, 522 aa, Unidentified
ETGHHHHHHQSPERPVFTCGGILTGESGFIGSEGFPGVYPPNSKCTWKITVPEGKVVVLNFRFIDLESDNLCRYDFVDVYNGHANGQRIGRFCGTFRPGALVSSGNKMMVQMISDANTAGNGFMAMFSAAEPNERGDQYCGGLLDRPSGSFKTPNWPDRDYPAGVTCVWHIVAPKNQLIELKFEKFDVERDNYCRYDYVAVFNGGEVNDARRIGKYCGDSPPAPIVSERNELLIQFLSDLSLTADGFIGHYIFRPKKLPTTTEQPVTTTFPVTTGLKPTVALASMVSKGEELFTGVVPILVELDGDVNGHKFSVSGEGEGDATYGKLTLKLICTTGKLPVPWPTLVTTLGYGLQCFARYPDHMKQHDFFKSAMPEGYVQERTIFFKDDGNYKTRAEVKFEGDTLVNRIELKGIDFKEDGNILGHKLEYNYNSHNVYITADKQKNGIKANFKIRHNIEDGGVQLADHYQQNTPIGDGPVLLPDNHYLSYQSKLSKDPNEKRDHMVLLEFVTAAGITLGMDELY

SEQ ID NO: 10 - protein, 640 aa, Unidentified
ETGTKIEEGKLVIWINGDKGYNGLAEVGKKFEKDTGIKVTVEHPDKLEEKFPQVAATGDGPDIIFWAHDRFGGYAQSGLLAEITPAAAFQDKLYPFTWDAVRYNGKLIAYPIAVEALSLIYNKDLLPNPPKTWEEIPALDKELKAKGKSALMFNLQEPYFTWPLIAADGGYAFKYAAGKYDIKDVGVDNAGAKAGLTFLVDLIKNKHMNADTDYSIAEHAFNHGETAMTINGPWAWSNIDTSAVNYGVTVLPTFKGQPSKPFVGVLSAGINAASPNKELAKEFLENYLLTDEGLEAVNKDKPLGAVALKSYEEELVKDPRVAATMENAQKGEIMPNIPQMSAFWYAVRTAVINAASGRQTVDAALAAAQTNAAALEVLFQGPASQSPERPVFTCGGILTGESGFIGSEGFPGVYPPNSKCTWKITVPEGKVVVLNFRFIDLESDNLCRYDFVDVYNGHANGQRIGRFCGTFRPGALVSSGNKMMVQMISDANTAGNGFMAMFSAAEPNERGDQYCGGLLDRPSGSFKTPNWPDRDYPAGVTCVWHIVAPKNQLIELKFEKFDVERDNYCRYDYVAVFNGGEVNDARRIGKYCGDSPPAPIVSERNELLIQFLSDLSLTADGFIGHYIFRPKKLEHHHHHH

SEQ ID NO: 11 - protein, 260 aa, Unidentified
GPASQSPERPVFTCGGILTGESGFIGSEGFPGVYPPNSKCTWKITVPEGKVVVLNFRFIDLESDNLCRYDFVDVYNGHANGQRIGRFCGTFRPGALVSSGNKMMVQMISDANTAGNGFMAMFSAAEPNERGDQYCGGLLDRPSGSFKTPNWPDRDYPAGVTCVWHIVAPKNQLIELKFEKFDVERDNYCRYDYVAVFNGGEVNDARRIGKYCGDSPPAPIVSERNELLIQFLSDLSLTADGFIGHYIFRPKKLEHHHHHH

SEQ ID NO: 12 - protein, 640 aa, Unidentified
ETGTKIEEGKLVIWINGDKGYNGLAEVGKKFEKDTGIKVTVEHPDKLEEKFPQVAATGDGPDIIFWAHDRFGGYAQSGLLAEITPAAAFQDKLYPFTWDAVRYNGKLIAYPIAVEALSLIYNKDLLPNPPKTWEEIPALDKELKAKGKSALMFNLQEPYFTWPLIAADGGYAFKYAAGKYDIKDVGVDNAGAKAGLTFLVDLIKNKHMNADTDYSIAEHAFNHGETAMTINGPWAWSNIDTSAVNYGVTVLPTFKGQPSKPFVGVLSAGINAASPNKELAKEFLENYLLTDEGLEAVNKDKPLGAVALKSYEEELVKDPRVAATMENAQKGEIMPNIPQMSAFWYAVRTAVINAASGRQTVDAALAAAQTNAAALEVLFQGPASQSPERPVFTCGGILTGESGFIGSEGFPGVYPPNSKCTWKITVPEGKVVVLNFRFIDLESDNLCRYDFVDVYNGHANGQRIGRFCGTARPGALVSSGNKMMVQMISDANTAGNGFMAMFSAAEPNERGDQYCGGLLDRPSGSFKTPNWPDRDYPAGVTCVWHIVAPKNQLIELKFEKFDVERDNYCRYDYVAVFNGGEVNDARRIGKYCGDSPPAPIVSERNELLIQFLSDLSLTADGFIGHYIFRPKKLEHHHHHH

SEQ ID NO: 13 - protein, 260 aa, Unidentified
GPASQSPERPVFTCGGILTGESGFIGSEGFPGVYPPNSKCTWKITVPEGKVVVLNFRFIDLESDNLCRYDFVDVYNGHANGQRIGRFCGTARPGALVSSGNKMMVQMISDANTAGNGFMAMFSAAEPNERGDQYCGGLLDRPSGSFKTPNWPDRDYPAGVTCVWHIVAPKNQLIELKFEKFDVERDNYCRYDYVAVFNGGEVNDARRIGKYCGDSPPAPIVSERNELLIQFLSDLSLTADGFIGHYIFRPKKLEHHHHHH

SEQ ID NO: 14 - protein, 640 aa, Unidentified
ETGTKIEEGKLVIWINGDKGYNGLAEVGKKFEKDTGIKVTVEHPDKLEEKFPQVAATGDGPDIIFWAHDRFGGYAQSGLLAEITPAAAFQDKLYPFTWDAVRYNGKLIAYPIAVEALSLIYNKDLLPNPPKTWEEIPALDKELKAKGKSALMFNLQEPYFTWPLIAADGGYAFKYAAGKYDIKDVGVDNAGAKAGLTFLVDLIKNKHMNADTDYSIAEHAFNHGETAMTINGPWAWSNIDTSAVNYGVTVLPTFKGQPSKPFVGVLSAGINAASPNKELAKEFLENYLLTDEGLEAVNKDKPLGAVALKSYEEELVKDPRVAATMENAQKGEIMPNIPQMSAFWYAVRTAVINAASGRQTVDAALAAAQTNAAALEVLFQGPASQSPERPVFTCGGILTGESGFIGSEGFPGVYPPNSKCTWKITVPEGKVVVLNFRFIDLESDNLCRYDFVDVYNGHANGQRIGRFCGTFDPGALVSSGNKMMVQMISDANTAGNGFMAMFSAAEPNERGDQYCGGLLDRPSGSFKTPNWPDRDYPAGVTCVWHIVAPKNQLIELKFEKFDVERDNYCRYDYVAVFNGGEVNDARRIGKYCGDSPPAPIVSERNELLIQFLSDLSLTADGFIGHYIFRPKKLEHHHHHH

SEQ ID NO: 15 - protein, 260 aa, Unidentified
GPASQSPERPVFTCGGILTGESGFIGSEGFPGVYPPNSKCTWKITVPEGKVVVLNFRFIDLESDNLCRYDFVDVYNGHANGQRIGRFCGTFDPGALVSSGNKMMVQMISDANTAGNGFMAMFSAAEPNERGDQYCGGLLDRPSGSFKTPNWPDRDYPAGVTCVWHIVAPKNQLIELKFEKFDVERDNYCRYDYVAVFNGGEVNDARRIGKYCGDSPPAPIVSERNELLIQFLSDLSLTADGFIGHYIFRPKKLEHHHHHH

SEQ ID NO: 16 - protein, 640 aa, Unidentified
ETGTKIEEGKLVIWINGDKGYNGLAEVGKKFEKDTGIKVTVEHPDKLEEKFPQVAATGDGPDIIFWAHDRFGGYAQSGLLAEITPAAAFQDKLYPFTWDAVRYNGKLIAYPIAVEALSLIYNKDLLPNPPKTWEEIPALDKELKAKGKSALMFNLQEPYFTWPLIAADGGYAFKYAAGKYDIKDVGVDNAGAKAGLTFLVDLIKNKHMNADTDYSIAEHAFNHGETAMTINGPWAWSNIDTSAVNYGVTVLPTFKGQPSKPFVGVLSAGINAASPNKELAKEFLENYLLTDEGLEAVNKDKPLGAVALKSYEEELVKDPRVAATMENAQKGEIMPNIPQMSAFWYAVRTAVINAASGRQTVDAALAAAQTNAAALEVLFQGPASQSPERPVFTCGGILTGESGFIGSEGFPGVYPPNSKCTWKITVPEGKVVVLNFRFIDLESDNLCRYDFVDVYNGHANGQRIGRFCGTFRPGALVSSGNKMMVQMISDANTAGNGFMAMFSAAEPNERGDQYCGGLLDRPSGSFKTPNWPDRDYPAGVTCVWHIVAPKNQLIELKFEKFDVERDNYCRYDYVAVFNGGEVNDARRIGKYCGDSPPAPIVSERNELLIQFLSDASLTADGFIGHYIFRPKKLEHHHHHH

SEQ ID NO: 17 - protein, 260 aa, Unidentified
GPASQSPERPVFTCGGILTGESGFIGSEGFPGVYPPNSKCTWKITVPEGKVVVLNFRFIDLESDNLCRYDFVDVYNGHANGQRIGRFCGTFRPGALVSSGNKMMVQMISDANTAGNGFMAMFSAAEPNERGDQYCGGLLDRPSGSFKTPNWPDRDYPAGVTCVWHIVAPKNQLIELKFEKFDVERDNYCRYDYVAVFNGGEVNDARRIGKYCGDSPPAPIVSERNELLIQFLSDASLTADGFIGHYIFRPKKLEHHHHHH

SEQ ID NO: 18 - protein, 640 aa, Unidentified
ETGTKIEEGKLVIWINGDKGYNGLAEVGKKFEKDTGIKVTVEHPDKLEEKFPQVAATGDGPDIIFWAHDRFGGYAQSGLLAEITPAAAFQDKLYPFTWDAVRYNGKLIAYPIAVEALSLIYNKDLLPNPPKTWEEIPALDKELKAKGKSALMFNLQEPYFTWPLIAADGGYAFKYAAGKYDIKDVGVDNAGAKAGLTFLVDLIKNKHMNADTDYSIAEHAFNHGETAMTINGPWAWSNIDTSAVNYGVTVLPTFKGQPSKPFVGVLSAGINAASPNKELAKEFLENYLLTDEGLEAVNKDKPLGAVALKSYEEELVKDPRVAATMENAQKGEIMPNIPQMSAFWYAVRTAVINAASGRQTVDAALAAAQTNAAALEVLFQGPASQSPERPVFTCGGILTGESGFIGSEGFPGVYPPNSKCTWKITVPEGKVVVLNFAFIDLESDNLCRYDFVDVYNGHANGQRIGRFCGTFRPGALVSSGNKMMVQMISDANTAGNGFMAMFSAAEPNERGDQYCGGLLDRPSGSFKTPNWPDRDYPAGVTCVWHIVAPKNQLIELKFEKFDVERDNYCRYDYVAVFNGGEVNDARRIGKYCGDSPPAPIVSERNELLIQFLSDASLTADGFIGHYIFRPKKLEHHHHHH

SEQ ID NO: 19 - protein, 260 aa, Unidentified
GPASQSPERPVFTCGGILTGESGFIGSEGFPGVYPPNSKCTWKITVPEGKVVVLNFAFIDLESDNLCRYDFVDVYNGHANGQRIGRFCGTFRPGALVSSGNKMMVQMISDANTAGNGFMAMFSAAEPNERGDQYCGGLLDRPSGSFKTPNWPDRDYPAGVTCVWHIVAPKNQLIELKFEKFDVERDNYCRYDYVAVFNGGEVNDARRIGKYCGDSPPAPIVSERNELLIQFLSDASLTADGFIGHYIFRPKKLEHHHHHH

SEQ ID NO: 20 - protein, 640 aa, Unidentified
ETGTKIEEGKLVIWINGDKGYNGLAEVGKKFEKDTGIKVTVEHPDKLEEKFPQVAATGDGPDIIFWAHDRFGGYAQSGLLAEITPAAAFQDKLYPFTWDAVRYNGKLIAYPIAVEALSLIYNKDLLPNPPKTWEEIPALDKELKAKGKSALMFNLQEPYFTWPLIAADGGYAFKYAAGKYDIKDVGVDNAGAKAGLTFLVDLIKNKHMNADTDYSIAEHAFNHGETAMTINGPWAWSNIDTSAVNYGVTVLPTFKGQPSKPFVGVLSAGINAASPNKELAKEFLENYLLTDEGLEAVNKDKPLGAVALKSYEEELVKDPRVAATMENAQKGEIMPNIPQMSAFWYAVRTAVINAASGRQTVDAALAAAQTNAAALEVLFQGPASQSPERPVFTCGGILTGESGFIGSEGFPGVYPPNSKCTWKITVPEGKVVVLNFAFIDLESDNLCRYDFVDVYNGHANGQRIGRFCGTADPGALVSSGNKMMVQMISDANTAGNGFMAMFSAAEPNERGDQYCGGLLDRPSGSFKTPNWPDRDYPAGVTCVWHIVAPKNQLIELKFEKFDVERDNYCRYDYVAVFNGGEVNDARRIGKYCGDSPPAPIVSERNELLIQFLSDASLTADGFIGHYIFRPKKLEHHHHHH

SEQ ID NO: 21 - protein, 260 aa, Unidentified
GPASQSPERPVFTCGGILTGESGFIGSEGFPGVYPPNSKCTWKITVPEGKVVVLNFAFIDLESDNLCRYDFVDVYNGHANGQRIGRFCGTADPGALVSSGNKMMVQMISDANTAGNGFMAMFSAAEPNERGDQYCGGLLDRPSGSFKTPNWPDRDYPAGVTCVWHIVAPKNQLIELKFEKFDVERDNYCRYDYVAVFNGGEVNDARRIGKYCGDSPPAPIVSERNELLIQFLSDASLTADGFIGHYIFRPKKLEHHHHHH

SEQ ID NO: 22 - protein, 271 aa, Unidentified
ETGHHHHHHCGGLLDRPSGSFKTPNWPDRDYPAGVTCVWHIVAPKNQLIELKFEKFDVERDNYCRYDYVAVFNGGEVNDARRIGKYCGDSPPAPIVSERNELLIQFLSDLSLTADGFIGHYIFRPKKLPTTTEQPVTTTFPVTTGLKPTVALCQQKCRRTGTLEGNYCSSDFVLAGTVITTITRDGSLHATVSIINIYKEGNLAIQQAGKNMSARLTVVCKQCPLLRRGLNYIIMGQVGEDGRGKIMPNSFIMMFKTKNQKLLDALKNKQC

SEQ ID NO: 23 - protein, 115 aa, Unidentified; identical to SEQ ID NO: 4

SEQ ID NO: 24 - protein, 112 aa, Unidentified; identical to SEQ ID NO: 1

SEQ ID NO: 25 - protein, 237 aa, Unidentified
CGGILTGESGFIGSEGFPGVYPPNSKCTWKITVPEGKVVVLNFRFIDLESDNLCRYDFVDVYNGHANGQRIGRFCGTFRPGALVSSGNKMMVQMISDANTAGNGFMAMFSAAGSGSGSGSGSCGGLLDRPSGSFKTPNWPDRDYPAGVTCVWHIVAPKNQLIELKFEKFDVERDNYCRYDYVAVFNGGEVNDARRIGKYCGDSPPAPIVSERNELLIQFLSDLSLTADGFIGHYIFR

SEQ ID NO: 26 - protein, 235 aa, Unidentified
CGGILTGESGFIGSEGFPGVYPPNSKCTWKITVPEGKVVVLNFRFIDLESDNLCRYDFVDVYNGHANGQRIGRFCGTFRPGALVSSGNKMMVQMISDANTAGNGFMAMFSAAGGGSGGGSCGGLLDRPSGSFKTPNWPDRDYPAGVTCVWHIVAPKNQLIELKFEKFDVERDNYCRYDYVAVFNGGEVNDARRIGKYCGDSPPAPIVSERNELLIQFLSDLSLTADGFIGHYIFR

SEQ ID NO: 27 - protein, 237 aa, Unidentified
CGGILTGESGFIGSEGFPGVYPPNSKCTWKITVPEGKVVVLNFRFIDLESDNLCRYDFVDVYNGHANGQRIGRFCGTARPGALVSSGNKMMVQMISDANTAGNGFMAMFSAAGSGSGSGSGSCGGLLDRPSGSFKTPNWPDRDYPAGVTCVWHIVAPKNQLIELKFEKFDVERDNYCRYDYVAVFNGGEVNDARRIGKYCGDSPPAPIVSERNELLIQFLSDLSLTADGFIGHYIFR

SEQ ID NO: 28 - protein, 235 aa, Unidentified
CGGILTGESGFIGSEGFPGVYPPNSKCTWKITVPEGKVVVLNFRFIDLESDNLCRYDFVDVYNGHANGQRIGRFCGTARPGALVSSGNKMMVQMISDANTAGNGFMAMFSAAGGGSGGGSCGGLLDRPSGSFKTPNWPDRDYPAGVTCVWHIVAPKNQLIELKFEKFDVERDNYCRYDYVAVFNGGEVNDARRIGKYCGDSPPAPIVSERNELLIQFLSDLSLTADGFIGHYIFR

SEQ ID NO: 29 - protein, 383 aa, Unidentified
CGGILTGESGFIGSEGFPGVYPPNSKCTWKITVPEGKVVVLNFRFIDLESDNLCRYDFVDVYNGHANGQRIGRFCGTFRPGALVSSGNKMMVQMISDANTAGNGFMAMFSAAEPNERGDQYCGGLLDRPSGSFKTPNWPDRDYPAGVTCVWHIVAPKNQLIELKFEKFDVERDNYCRYDYVAVFNGGEVNDARRIGKYCGDSPPAPIVSERNELLIQFLSDLSLTADGFIGHYIFRPKKLPTTTEQPVTTTFPVTTGLKPTVALCQQKCRRTGTLEGNYCSSDFVLAGTVITTITRDGSLHATVSIINIYKEGNLAIQQAGKNMSARLTVVCKQCPLLRRGLNYIIMGQVGEDGRGKIMPNSFIMMFKTKNQKLLDALKNKQC

SEQ ID NO: 30 - protein, 391 aa, Unidentified
CGGILTGESGFIGSEGFPGVYPPNSKCTWKITVPEGKVVVLNFRFIDLESDNLCRYDFVDVYNGHANGQRIGRFCGTFRPGALVSSGNKMMVQMISDANTAGNGFMAMFSAAEPNERGDQYCGGLLDRPSGSFKTPNWPDRDYPAGVTCVWHIVAPKNQLIELKFEKFDVERDNYCRYDYVAVFNGGEVNDARRIGKYCGDSPPAPIVSERNELLIQFLSDLSLTADGFIGHYIFRPKLEVLFQGPKLPTTTEQPVTTTFPVTTGLKPTVALCQQKCRRTGTLEGNYCSSDFVLAGTVITTITRDGSLHATVSIINIYKEGNLAIQQAGKNMSARLTVVCKQCPLLRRGLNYIIMGQVGEDGRGKIMPNSFIMMFKTKNQKLLDALKNKQC

SEQ ID NO: 31 - protein, 504 aa, Unidentified
CGGILTGESGFIGSEGFPGVYPPNSKCTWKITVPEGKVVVLNFRFIDLESDNLCRYDFVDVYNGHANGQRIGRFCGTFRPGALVSSGNKMMVQMISDANTAGNGFMAMFSAAEPNERGDQYCGGLLDRPSGSFKTPNWPDRDYPAGVTCVWHIVAPKNQLIELKFEKFDVERDNYCRYDYVAVFNGGEVNDARRIGKYCGDSPPAPIVSERNELLIQFLSDLSLTADGFIGHYIFRPKKLPTTTEQPVTTTFPVTTGLKPTVALASMVSKGEELFTGVVPILVELDGDVNGHKFSVSGEGEGDATYGKLTLKLICTTGKLPVPWPTLVTTLGYGLQCFARYPDHMKQHDFFKSAMPEGYVQERTIFFKDDGNYKTRAEVKFEGDTLVNRIELKGIDFKEDGNILGHKLEYNYNSHNVYITADKQKNGIKANFKIRHNIEDGGVQLADHYQQNTPIGDGPVLLPDNHYLSYQSKLSKDPNEKRDHMVLLEFVTAAGITLGMDELY

SEQ ID NO: 32 - protein, 629 aa, Unidentified
KIEEGKLVIWINGDKGYNGLAEVGKKFEKDTGIKVTVEHPDKLEEKFPQVAATGDGPDIIFWAHDRFGGYAQSGLLAEITPAAAFQDKLYPFTWDAVRYNGKLIAYPIAVEALSLIYNKDLLPNPPKTWEEIPALDKELKAKGKSALMFNLQEPYFTWPLIAADGGYAFKYAAGKYDIKDVGVDNAGAKAGLTFLVDLIKNKHMNADTDYSIAEHAFNHGETAMTINGPWAWSNIDTSAVNYGVTVLPTFKGQPSKPFVGVLSAGINAASPNKELAKEFLENYLLTDEGLEAVNKDKPLGAVALKSYEEELVKDPRVAATMENAQKGEIMPNIPQMSAFWYAVRTAVINAASGRQTVDAALAAAQTNAAALEVLFQGPASQSPERPVFTCGGILTGESGFIGSEGFPGVYPPNSKCTWKITVPEGKVVVLNFRFIDLESDNLCRYDFVDVYNGHANGQRIGRFCGTFRPGALVSSGNKMMVQMISDANTAGNGFMAMFSAAEPNERGDQYCGGLLDRPSGSFKTPNWPDRDYPAGVTCVWHIVAPKNQLIELKFEKFDVERDNYCRYDYVAVFNGGEVNDARRIGKYCGDSPPAPIVSERNELLIQFLSDLSLTADGFIGHYIFRPKKL

SEQ ID NO: 33 - protein, 625 aa, Unidentified
KIEEGKLVIWINGDKGYNGLAEVGKKFEKDTGIKVTVEHPDKLEEKFPQVAATGDGPDIIFWAHDRFGGYAQSGLLAEITPAAAFQDKLYPFTWDAVRYNGKLIAYPIAVEALSLIYNKDLLPNPPKTWEEIPALDKELKAKGKSALMFNLQEPYFTWPLIAADGGYAFKYAAGKYDIKDVGVDNAGAKAGLTFLVDLIKNKHMNADTDYSIAEHAFNHGETAMTINGPWAWSNIDTSAVNYGVTVLPTFKGQPSKPFVGVLSAGINAASPNKELAKEFLENYLLTDEGLEAVNKDKPLGAVALKSYEEELVKDPRVAATMENAQKGEIMPNIPQMSAFWYAVRTAVINAASGRQTVDAALAAAQTNAAALEVLFQGPASQSPERPVFTCGGILTGESGFIGSEGFPGVYPPNSKCTWKITVPEGKVVVLNFRFIDLESDNLCRYDFVDVYNGHANGQRIGRFCGTFRPGALVSSGNKMMVQMISDANTAGNGFMAMFSAAEPNERGDQYCGGLLDRPSGSFKTPNWPDRDYPAGVTCVWHIVAPKNQLIELKFEKFDVERDNYCRYDYVAVFNGGEVNDARRIGKYCGDSPPAPIVSERNELLIQFLSDLSLTADGFIGHYIFR

SEQ ID NO: 34 - protein, 240 aa, Unidentified
CGGILTGESGFIGSEGFPGVYPPNSKCTWKITVPEGKVVVLNFRFIDLESDNLCRYDFVDVYNGHANGQRIGRFCGTFRPGALVSSGNKMMVQMISDANTAGNGFMAMFSAAEPNERGDQYCGGLLDRPSGSFKTPNWPDRDYPAGVTCVWHIVAPKNQLIELKFEKFDVERDNYCRYDYVAVFNGGEVNDARRIGKYCGDSPPAPIVSERNELLIQFLSDLSLTADGFIGHYIFRPKKL

SEQ ID NO: 35 - protein, 236 aa, Unidentified
CGGILTGESGFIGSEGFPGVYPPNSKCTWKITVPEGKVVVLNFRFIDLESDNLCRYDFVDVYNGHANGQRIGRFCGTFRPGALVSSGNKMMVQMISDANTAGNGFMAMFSAAEPNERGDQYCGGLLDRPSGSFKTPNWPDRDYPAGVTCVWHIVAPKNQLIELKFEKFDVERDNYCRYDYVAVFNGGEVNDARRIGKYCGDSPPAPIVSERNELLIQFLSDLSLTADGFIGHYIFR

SEQ ID NO: 36 - protein, 629 aa, Unidentified
KIEEGKLVIWINGDKGYNGLAEVGKKFEKDTGIKVTVEHPDKLEEKFPQVAATGDGPDIIFWAHDRFGGYAQSGLLAEITPAAAFQDKLYPFTWDAVRYNGKLIAYPIAVEALSLIYNKDLLPNPPKTWEEIPALDKELKAKGKSALMFNLQEPYFTWPLIAADGGYAFKYAAGKYDIKDVGVDNAGAKAGLTFLVDLIKNKHMNADTDYSIAEHAFNHGETAMTINGPWAWSNIDTSAVNYGVTVLPTFKGQPSKPFVGVLSAGINAASPNKELAKEFLENYLLTDEGLEAVNKDKPLGAVALKSYEEELVKDPRVAATMENAQKGEIMPNIPQMSAFWYAVRTAVINAASGRQTVDAALAAAQTNAAALEVLFQGPASQSPERPVFTCGGILTGESGFIGSEGFPGVYPPNSKCTWKITVPEGKVVVLNFRFIDLESDNLCRYDFVDVYNGHANGQRIGRFCGTARPGALVSSGNKMMVQMISDANTAGNGFMAMFSAAEPNERGDQYCGGLLDRPSGSFKTPNWPDRDYPAGVTCVWHIVAPKNQLIELKFEKFDVERDNYCRYDYVAVFNGGEVNDARRIGKYCGDSPPAPIVSERNELLIQFLSDLSLTADGFIGHYIFRPKKL

SEQ ID NO: 37 - protein, 625 aa, Unidentified
KIEEGKLVIWINGDKGYNGLAEVGKKFEKDTGIKVTVEHPDKLEEKFPQVAATGDGPDIIFWAHDRFGGYAQSGLLAEITPAAAFQDKLYPFTWDAVRYNGKLIAYPIAVEALSLIYNKDLLPNPPKTWEEIPALDKELKAKGKSALMFNLQEPYFTWPLIAADGGYAFKYAAGKYDIKDVGVDNAGAKAGLTFLVDLIKNKHMNADTDYSIAEHAFNHGETAMTINGPWAWSNIDTSAVNYGVTVLPTFKGQPSKPFVGVLSAGINAASPNKELAKEFLENYLLTDEGLEAVNKDKPLGAVALKSYEEELVKDPRVAATMENAQKGEIMPNIPQMSAFWYAVRTAVINAASGRQTVDAALAAAQTNAAALEVLFQGPASQSPERPVFTCGGILTGESGFIGSEGFPGVYPPNSKCTWKITVPEGKVVVLNFRFIDLESDNLCRYDFVDVYNGHANGQRIGRFCGTARPGALVSSGNKMMVQMISDANTAGNGFMAMFSAAEPNERGDQYCGGLLDRPSGSFKTPNWPDRDYPAGVTCVWHIVAPKNQLIELKFEKFDVERDNYCRYDYVAVFNGGEVNDARRIGKYCGDSPPAPIVSERNELLIQFLSDLSLTADGFIGHYIFR

SEQ ID NO: 38 - protein, 240 aa, Unidentified
CGGILTGESGFIGSEGFPGVYPPNSKCTWKITVPEGKVVVLNFRFIDLESDNLCRYDFVDVYNGHANGQRIGRFCGTARPGALVSSGNKMMVQMISDANTAGNGFMAMFSAAEPNERGDQYCGGLLDRPSGSFKTPNWPDRDYPAGVTCVWHIVAPKNQLIELKFEKFDVERDNYCRYDYVAVFNGGEVNDARRIGKYCGDSPPAPIVSERNELLIQFLSDLSLTADGFIGHYIFRPKKL

SEQ ID NO: 39 - protein, 236 aa, Unidentified
CGGILTGESGFIGSEGFPGVYPPNSKCTWKITVPEGKVVVLNFRFIDLESDNLCRYDFVDVYNGHANGQRIGRFCGTARPGALVSSGNKMMVQMISDANTAGNGFMAMFSAAEPNERGDQYCGGLLDRPSGSFKTPNWPDRDYPAGVTCVWHIVAPKNQLIELKFEKFDVERDNYCRYDYVAVFNGGEVNDARRIGKYCGDSPPAPIVSERNELLIQFLSDLSLTADGFIGHYIFR

SEQ ID NO: 40 - protein, 629 aa, Unidentified
KIEEGKLVIWINGDKGYNGLAEVGKKFEKDTGIKVTVEHPDKLEEKFPQVAATGDGPDIIFWAHDRFGGYAQSGLLAEITPAAAFQDKLYPFTWDAVRYNGKLIAYPIAVEALSLIYNKDLLPNPPKTWEEIPALDKELKAKGKSALMFNLQEPYFTWPLIAADGGYAFKYAAGKYDIKDVGVDNAGAKAGLTFLVDLIKNKHMNADTDYSIAEHAFNHGETAMTINGPWAWSNIDTSAVNYGVTVLPTFKGQPSKPFVGVLSAGINAASPNKELAKEFLENYLLTDEGLEAVNKDKPLGAVALKSYEEELVKDPRVAATMENAQKGEIMPNIPQMSAFWYAVRTAVINAASGRQTVDAALAAAQTNAAALEVLFQGPASQSPERPVFTCGGILTGESGFIGSEGFPGVYPPNSKCTWKITVPEGKVVVLNFRFIDLESDNLCRYDFVDVYNGHANGQRIGRFCGTFDPGALVSSGNKMMVQMISDANTAGNGFMAMFSAAEPNERGDQYCGGLLDRPSGSFKTPNWPDRDYPAGVTCVWHIVAPKNQLIELKFEKFDVERDNYCRYDYVAVFNGGEVNDARRIGKYCGDSPPAPIVSERNELLIQFLSDLSLTADGFIGHYIFRPKKL

SEQ ID NO: 41 - protein, 625 aa, Unidentified
KIEEGKLVIWINGDKGYNGLAEVGKKFEKDTGIKVTVEHPDKLEEKFPQVAATGDGPDIIFWAHDRFGGYAQSGLLAEITPAAAFQDKLYPFTWDAVRYNGKLIAYPIAVEALSLIYNKDLLPNPPKTWEEIPALDKELKAKGKSALMFNLQEPYFTWPLIAADGGYAFKYAAGKYDIKDVGVDNAGAKAGLTFLVDLIKNKHMNADTDYSIAEHAFNHGETAMTINGPWAWSNIDTSAVNYGVTVLPTFKGQPSKPFVGVLSAGINAASPNKELAKEFLENYLLTDEGLEAVNKDKPLGAVALKSYEEELVKDPRVAATMENAQKGEIMPNIPQMSAFWYAVRTAVINAASGRQTVDAALAAAQTNAAALEVLFQGPASQSPERPVFTCGGILTGESGFIGSEGFPGVYPPNSKCTWKITVPEGKVVVLNFRFIDLESDNLCRYDFVDVYNGHANGQRIGRFCGTFDPGALVSSGNKMMVQMISDANTAGNGFMAMFSAAEPNERGDQYCGGLLDRPSGSFKTPNWPDRDYPAGVTCVWHIVAPKNQLIELKFEKFDVERDNYCRYDYVAVFNGGEVNDARRIGKYCGDSPPAPIVSERNELLIQFLSDLSLTADGFIGHYIFR

SEQ ID NO: 42 - protein, 240 aa, Unidentified
CGGILTGESGFIGSEGFPGVYPPNSKCTWKITVPEGKVVVLNFRFIDLESDNLCRYDFVDVYNGHANGQRIGRFCGTFDPGALVSSGNKMMVQMISDANTAGNGFMAMFSAAEPNERGDQYCGGLLDRPSGSFKTPNWPDRDYPAGVTCVWHIVAPKNQLIELKFEKFDVERDNYCRYDYVAVFNGGEVNDARRIGKYCGDSPPAPIVSERNELLIQFLSDLSLTADGFIGHYIFRPKKL

SEQ ID NO: 43 - protein, 236 aa, Unidentified
CGGILTGESGFIGSEGFPGVYPPNSKCTWKITVPEGKVVVLNFRFIDLESDNLCRYDFVDVYNGHANGQRIGRFCGTFDPGALVSSGNKMMVQMISDANTAGNGFMAMFSAAEPNERGDQYCGGLLDRPSGSFKTPNWPDRDYPAGVTCVWHIVAPKNQLIELKFEKFDVERDNYCRYDYVAVFNGGEVNDARRIGKYCGDSPPAPIVSERNELLIQFLSDLSLTADGFIGHYIFR

SEQ ID NO: 44 - protein, 629 aa, Unidentified
KIEEGKLVIWINGDKGYNGLAEVGKKFEKDTGIKVTVEHPDKLEEKFPQVAATGDGPDIIFWAHDRFGGYAQSGLLAEITPAAAFQDKLYPFTWDAVRYNGKLIAYPIAVEALSLIYNKDLLPNPPKTWEEIPALDKELKAKGKSALMFNLQEPYFTWPLIAADGGYAFKYAAGKYDIKDVGVDNAGAKAGLTFLVDLIKNKHMNADTDYSIAEHAFNHGETAMTINGPWAWSNIDTSAVNYGVTVLPTFKGQPSKPFVGVLSAGINAASPNKELAKEFLENYLLTDEGLEAVNKDKPLGAVALKSYEEELVKDPRVAATMENAQKGEIMPNIPQMSAFWYAVRTAVINAASGRQTVDAALAAAQTNAAALEVLFQGPASQSPERPVFTCGGILTGESGFIGSEGFPGVYPPNSKCTWKITVPEGKVVVLNFRFIDLESDNLCRYDFVDVYNGHANGQRIGRFCGTFRPGALVSSGNKMMVQMISDANTAGNGFMAMFSAAEPNERGDQYCGGLLDRPSGSFKTPNWPDRDYPAGVTCVWHIVAPKNQLIELKFEKFDVERDNYCRYDYVAVFNGGEVNDARRIGKYCGDSPPAPIVSERNELLIQFLSDASLTADGFIGHYIFRPKKL

SEQ ID NO: 45 - protein, 625 aa, Unidentified
KIEEGKLVIWINGDKGYNGLAEVGKKFEKDTGIKVTVEHPDKLEEKFPQVAATGDGPDIIFWAHDRFGGYAQSGLLAEITPAAAFQDKLYPFTWDAVRYNGKLIAYPIAVEALSLIYNKDLLPNPPKTWEEIPALDKELKAKGKSALMFNLQEPYFTWPLIAADGGYAFKYAAGKYDIKDVGVDNAGAKAGLTFLVDLIKNKHMNADTDYSIAEHAFNHGETAMTINGPWAWSNIDTSAVNYGVTVLPTFKGQPSKPFVGVLSAGINAASPNKELAKEFLENYLLTDEGLEAVNKDKPLGAVALKSYEEELVKDPRVAATMENAQKGEIMPNIPQMSAFWYAVRTAVINAASGRQTVDAALAAAQTNAAALEVLFQGPASQSPERPVFTCGGILTGESGFIGSEGFPGVYPPNSKCTWKITVPEGKVVVLNFRFIDLESDNLCRYDFVDVYNGHANGQRIGRFCGTFRPGALVSSGNKMMVQMISDANTAGNGFMAMFSAAEPNERGDQYCGGLLDRPSGSFKTPNWPDRDYPAGVTCVWHIVAPKNQLIELKFEKFDVERDNYCRYDYVAVFNGGEVNDARRIGKYCGDSPPAPIVSERNELLIQFLSDASLTADGFIGHYIFR

SEQ ID NO: 46 - protein, 240 aa, Unidentified
CGGILTGESGFIGSEGFPGVYPPNSKCTWKITVPEGKVVVLNFRFIDLESDNLCRYDFVDVYNGHANGQRIGRFCGTFRPGALVSSGNKMMVQMISDANTAGNGFMAMFSAAEPNERGDQYCGGLLDRPSGSFKTPNWPDRDYPAGVTCVWHIVAPKNQLIELKFEKFDVERDNYCRYDYVAVFNGGEVNDARRIGKYCGDSPPAPIVSERNELLIQFLSDASLTADGFIGHYIFRPKKL

SEQ ID NO: 47 - protein, 236 aa, Unidentified
CGGILTGESGFIGSEGFPGVYPPNSKCTWKITVPEGKVVVLNFRFIDLESDNLCRYDFVDVYNGHANGQRIGRFCGTFRPGALVSSGNKMMVQMISDANTAGNGFMAMFSAAEPNERGDQYCGGLLDRPSGSFKTPNWPDRDYPAGVTCVWHIVAPKNQLIELKFEKFDVERDNYCRYDYVAVFNGGEVNDARRIGKYCGDSPPAPIVSERNELLIQFLSDASLTADGFIGHYIFR

SEQ ID NO: 48 - protein, 629 aa, Unidentified
KIEEGKLVIWINGDKGYNGLAEVGKKFEKDTGIKVTVEHPDKLEEKFPQVAATGDGPDIIFWAHDRFGGYAQSGLLAEITPAAAFQDKLYPFTWDAVRYNGKLIAYPIAVEALSLIYNKDLLPNPPKTWEEIPALDKELKAKGKSALMFNLQEPYFTWPLIAADGGYAFKYAAGKYDIKDVGVDNAGAKAGLTFLVDLIKNKHMNADTDYSIAEHAFNHGETAMTINGPWAWSNIDTSAVNYGVTVLPTFKGQPSKPFVGVLSAGINAASPNKELAKEFLENYLLTDEGLEAVNKDKPLGAVALKSYEEELVKDPRVAATMENAQKGEIMPNIPQMSAFWYAVRTAVINAASGRQTVDAALAAAQTNAAALEVLFQGPASQSPERPVFTCGGILTGESGFIGSEGFPGVYPPNSKCTWKITVPEGKVVVLNFAFIDLESDNLCRYDFVDVYNGHANGQRIGRFCGTFRPGALVSSGNKMMVQMISDANTAGNGFMAMFSAAEPNERGDQYCGGLLDRPSGSFKTPNWPDRDYPAGVTCVWHIVAPKNQLIELKFEKFDVERDNYCRYDYVAVFNGGEVNDARRIGKYCGDSPPAPIVSERNELLIQFLSDASLTADGFIGHYIFRPKKL

SEQ ID NO: 49 - protein, 625 aa, Unidentified
KIEEGKLVIWINGDKGYNGLAEVGKKFEKDTGIKVTVEHPDKLEEKFPQVAATGDGPDIIFWAHDRFGGYAQSGLLAEITPAAAFQDKLYPFTWDAVRYNGKLIAYPIAVEALSLIYNKDLLPNPPKTWEEIPALDKELKAKGKSALMFNLQEPYFTWPLIAADGGYAFKYAAGKYDIKDVGVDNAGAKAGLTFLVDLIKNKHMNADTDYSIAEHAFNHGETAMTINGPWAWSNIDTSAVNYGVTVLPTFKGQPSKPFVGVLSAGINAASPNKELAKEFLENYLLTDEGLEAVNKDKPLGAVALKSYEEELVKDPRVAATMENAQKGEIMPNIPQMSAFWYAVRTAVINAASGRQTVDAALAAAQTNAAALEVLFQGPASQSPERPVFTCGGILTGESGFIGSEGFPGVYPPNSKCTWKITVPEGKVVVLNFAFIDLESDNLCRYDFVDVYNGHANGQRIGRFCGTFRPGALVSSGNKMMVQMISDANTAGNGFMAMFSAAEPNERGDQYCGGLLDRPSGSFKTPNWPDRDYPAGVTCVWHIVAPKNQLIELKFEKFDVERDNYCRYDYVAVFNGGEVNDARRIGKYCGDSPPAPIVSERNELLIQFLSDASLTADGFIGHYIFR

SEQ ID NO: 50 - protein, 240 aa, Unidentified
CGGILTGESGFIGSEGFPGVYPPNSKCTWKITVPEGKVVVLNFAFIDLESDNLCRYDFVDVYNGHANGQRIGRFCGTFRPGALVSSGNKMMVQMISDANTAGNGFMAMFSAAEPNERGDQYCGGLLDRPSGSFKTPNWPDRDYPAGVTCVWHIVAPKNQLIELKFEKFDVERDNYCRYDYVAVFNGGEVNDARRIGKYCGDSPPAPIVSERNELLIQFLSDASLTADGFIGHYIFRPKKL

SEQ ID NO: 51 - protein, 236 aa, Unidentified
CGGILTGESGFIGSEGFPGVYPPNSKCTWKITVPEGKVVVLNFAFIDLESDNLCRYDFVDVYNGHANGQRIGRFCGTFRPGALVSSGNKMMVQMISDANTAGNGFMAMFSAAEPNERGDQYCGGLLDRPSGSFKTPNWPDRDYPAGVTCVWHIVAPKNQLIELKFEKFDVERDNYCRYDYVAVFNGGEVNDARRIGKYCGDSPPAPIVSERNELLIQFLSDASLTADGFIGHYIFR

SEQ ID NO: 52 - protein, 629 aa, Unidentified
KIEEGKLVIWINGDKGYNGLAEVGKKFEKDTGIKVTVEHPDKLEEKFPQVAATGDGPDIIFWAHDRFGGYAQSGLLAEITPAAAFQDKLYPFTWDAVRYNGKLIAYPIAVEALSLIYNKDLLPNPPKTWEEIPALDKELKAKGKSALMFNLQEPYFTWPLIAADGGYAFKYAAGKYDIKDVGVDNAGAKAGLTFLVDLIKNKHMNADTDYSIAEHAFNHGETAMTINGPWAWSNIDTSAVNYGVTVLPTFKGQPSKPFVGVLSAGINAASPNKELAKEFLENYLLTDEGLEAVNKDKPLGAVALKSYEEELVKDPRVAATMENAQKGEIMPNIPQMSAFWYAVRTAVINAASGRQTVDAALAAAQTNAAALEVLFQGPASQSPERPVFTCGGILTGESGFIGSEGFPGVYPPNSKCTWKITVPEGKVVVLNFAFIDLESDNLCRYDFVDVYNGHANGQRIGRFCGTADPGALVSSGNKMMVQMISDANTAGNGFMAMFSAAEPNERGDQYCGGLLDRPSGSFKTPNWPDRDYPAGVTCVWHIVAPKNQLIELKFEKFDVERDNYCRYDYVAVFNGGEVNDARRIGKYCGDSPPAPIVSERNELLIQFLSDASLTADGFIGHYIFRPKKL

SEQ ID NO: 53 - protein, 625 aa, Unidentified
KIEEGKLVIWINGDKGYNGLAEVGKKFEKDTGIKVTVEHPDKLEEKFPQVAATGDGPDIIFWAHDRFGGYAQSGLLAEITPAAAFQDKLYPFTWDAVRYNGKLIAYPIAVEALSLIYNKDLLPNPPKTWEEIPALDKELKAKGKSALMFNLQEPYFTWPLIAADGGYAFKYAAGKYDIKDVGVDNAGAKAGLTFLVDLIKNKHMNADTDYSIAEHAFNHGETAMTINGPWAWSNIDTSAVNYGVTVLPTFKGQPSKPFVGVLSAGINAASPNKELAKEFLENYLLTDEGLEAVNKDKPLGAVALKSYEEELVKDPRVAATMENAQKGEIMPNIPQMSAFWYAVRTAVINAASGRQTVDAALAAAQTNAAALEVLFQGPASQSPERPVFTCGGILTGESGFIGSEGFPGVYPPNSKCTWKITVPEGKVVVLNFAFIDLESDNLCRYDFVDVYNGHANGQRIGRFCGTADPGALVSSGNKMMVQMISDANTAGNGFMAMFSAAEPNERGDQYCGGLLDRPSGSFKTPNWPDRDYPAGVTCVWHIVAPKNQLIELKFEKFDVERDNYCRYDYVAVFNGGEVNDARRIGKYCGDSPPAPIVSERNELLIQFLSDASLTADGFIGHYIFR

SEQ ID NO: 54 - protein, 240 aa, Unidentified
CGGILTGESGFIGSEGFPGVYPPNSKCTWKITVPEGKVVVLNFAFIDLESDNLCRYDFVDVYNGHANGQRIGRFCGTADPGALVSSGNKMMVQMISDANTAGNGFMAMFSAAEPNERGDQYCGGLLDRPSGSFKTPNWPDRDYPAGVTCVWHIVAPKNQLIELKFEKFDVERDNYCRYDYVAVFNGGEVNDARRIGKYCGDSPPAPIVSERNELLIQFLSDASLTADGFIGHYIFRPKKL

SEQ ID NO: 55 - protein, 236 aa, Unidentified
CGGILTGESGFIGSEGFPGVYPPNSKCTWKITVPEGKVVVLNFAFIDLESDNLCRYDFVDVYNGHANGQRIGRFCGTADPGALVSSGNKMMVQMISDANTAGNGFMAMFSAAEPNERGDQYCGGLLDRPSGSFKTPNWPDRDYPAGVTCVWHIVAPKNQLIELKFEKFDVERDNYCRYDYVAVFNGGEVNDARRIGKYCGDSPPAPIVSERNELLIQFLSDASLTADGFIGHYIFR

SEQ ID NO: 56 - protein, 262 aa, Unidentified
CGGLLDRPSGSFKTPNWPDRDYPAGVTCVWHIVAPKNQLIELKFEKFDVERDNYCRYDYVAVFNGGEVNDARRIGKYCGDSPPAPIVSERNELLIQFLSDLSLTADGFIGHYIFRPKKLPTTTEQPVTTTFPVTTGLKPTVALCQQKCRRTGTLEGNYCSSDFVLAGTVITTITRDGSLHATVSIINIYKEGNLAIQQAGKNMSARLTVVCKQCPLLRRGLNYIIMGQVGEDGRGKIMPNSFIMMFKTKNQKLLDALKNKQC

SEQ ID NO: 57 - protein, 247 aa, Unidentified
CGGLLDRPSGSFKTPNWPDRDYPAGVTCVWHIVAPKNQLIELKFEKFDVERDNYCRYDYVAVFNGGEVNDARRIGKYCGDSPPAPIVSERNELLIQFLSDLSLTADGFIGHYIFRGSGSGSGSGSGSGSGSGSGSCGGILTGESGFIGSEGFPGVYPPNSKCTWKITVPEGKVVVLNFRFIDLESDNLCRYDFVDVYNGHANGQRIGRFCGTFRPGALVSSGNKMMVQMISDANTAGNGFMAMFSAA

SEQ ID NO: 58 - protein, 236 aa, Unidentified
CGGILTGESGFIGSEGFPGVYPPNSKCTWKITVPEGKVVVLNFRFIDLESDNLCRYDFVDVYNGHANGQRIGRFCGTFRPGALVSSGNKMMVQMISDANTAGNGFMAMFSAAATSGTEHQFCGGLLDRPSGSFKTPNWPDRDYPAGVTCVWHIVAPKNQLIELKFEKFDVERDNYCRYDYVAVFNGGEVNDARRIGKYCGDSPPAPIVSERNELLIQFLSDLSLTADGFIGHYIFR

SEQ ID NO: 59 - protein, 240 aa, Unidentified
CGGILTGESGFIGSEGFPGVYPPNSKCTWKITVPEGKVVVLNFRFIDLESHNLCRYDFVDVYNGHANGQRIGRFCGTARPGALVSSGNKMMVQMISDANTAGNGFMAMFSAAEPNERGDQYCGGLLDRPSGSFKTPNWPDRDYPAGVTCVWHIVAPKNQLIELKFEKFDVERHDYCRYDYVAVFNGGEVNDARRIGKYCGDSPPAPIVSERNELLIQFLSDLSLTADGFIGHYIFRPKKL

SEQ ID NO: 60 - protein, 248 aa, Homo sapiens
QTPNYTRPVFLCGGDVKGESGYVASEGFPNLYPPNKECIWTITVPEGQTVSLSFRVFDLELHPACRYDALEVFAGSGTSGQRLGRFCGTFRPAPLVAPGNQVTLRMTTDEGTGGRGFLLWYSGRATSGTEHQFCGGRLEKAQGTLTTPNWPESDYPPGISCSWHIIAPPDQVIALTFEKFDLEPDTYCRYDSVSVFNGAVSDDSRRLGKFCGDAVPGSISSEGNELLVQFVSDLSVTADGFSASYKTL

SEQ ID NO: 61 - protein, 245 aa, Homo sapiens
QSPERPVFTCGGILTGESGFIGSEGFPGVYPPNSKCTWKITVPEGKVVVLNFRFIDLESDNLCRYDFVDVYNGHANGQRIGRFCGTFRPGALVSSGNKMMVQMISDANTAGNGFMAMFSAAEPNERGDQYCGGLLDRPSGSFKTPNWPDRDYPAGVTCVWHIVAPKNQLIELKFEKFDVERDNYCRYDYVAVFNGGEVNDARRIGKYCGDSPPAPIVSERNELLIQFLSDLSLTADGFIGHYIFR

SEQ ID NO: 62 - protein, 30 aa, Unidentified
DVERDNYCRYDYVAVFNGGEVNDARRIGKY

SEQ ID NO: 63 - protein, 16 aa, unidentified
FRPKLEVLFQGPKLPT

SEQ ID NO: 64 - protein, 18 aa, unidentified
ETGHHHHHHLEVLFSPAS